European Patent Application EP 4 759 935 A1, published June 17, 2026. Title: Straight-chain inulin synthetic bacterium and method for producing straight-chain inulin. Applicant: 日本甜菜製糖株式会社. The sequence listing filed with the application follows.

SEQUENCE LISTING (49 sequences)

SEQ ID NO: 1 - DNA, 33 bp, synthetic construct
  misc_feature 1..33: note = 928-3_IS_s
  source 1..33: mol_type = other DNA
ggagatatacatatgtttgcagcggaaatcagt

SEQ ID NO: 2 - DNA, 33 bp, synthetic construct
  misc_feature 1..33: note = 928-3_IS_as
  source 1..33: mol_type = other DNA
gtggtggtggtggtggcgatttgccccaaatgg

SEQ ID NO: 3 - DNA, 33 bp, synthetic construct
  misc_feature 1..33: note = 928-3_ORF1_s
  source 1..33: mol_type = other DNA
ggagatatacatatggaagacgtagggcaaacg

SEQ ID NO: 4 - DNA, 33 bp, synthetic construct
  misc_feature 1..33: note = 928-3_ORF1_as
  source 1..33: mol_type = other DNA
gtggtggtggtggtgttgtttaatccagccagg

SEQ ID NO: 5 - DNA, 32 bp, synthetic construct
  misc_feature 1..32: note = Sma1-IS_s
  source 1..32: mol_type = other DNA
aaaaacccgggaacccattccgttcctgcagg

SEQ ID NO: 6 - DNA, 35 bp, synthetic construct
  misc_feature 1..35: note = Sma1-IS_as
  source 1..35: mol_type = other DNA
cggtcaaatcatttccttagcgatttgccccaaat

SEQ ID NO: 7 - DNA, 19 bp, synthetic construct
  misc_feature 1..19: note = ORF3-Xba1_s
  source 1..19: mol_type = other DNA
taaggaaatgatttgaccg

SEQ ID NO: 8 - DNA, 31 bp, synthetic construct
  misc_feature 1..31: note = ORF3-Xba1_as
  source 1..31: mol_type = other DNA
aaaaatctagagatcatggcgttttccagga

SEQ ID NO: 9 - DNA, 18 bp, synthetic construct
  misc_feature 1..18: note = pHY300_UP1
  source 1..18: mol_type = other DNA
tcattagttggctggtta

SEQ ID NO: 10 - DNA, 21 bp, synthetic construct
  misc_feature 1..21: note = BI_start_as
  source 1..21: mol_type = other DNA
attcataacggtcatccttct

SEQ ID NO: 11 - DNA, 33 bp, synthetic construct
  misc_feature 1..33: note = WP_099354679.1_s
  source 1..33: mol_type = other DNA
ggagatatacatatggcagaaacagaggtaacg

SEQ ID NO: 12 - DNA, 33 bp, synthetic construct
  misc_feature 1..33: note = WP_099354679.1_as
  source 1..33: mol_type = other DNA
gtggtggtggtggtgttgcttaatccaaccagg

SEQ ID NO: 13 - DNA, 33 bp, synthetic construct
  misc_feature 1..33: note = SHR63422.1_s
  source 1..33: mol_type = other DNA
ggagatatacatatggatgaaaccgtaacgacc

SEQ ID NO: 14 - DNA, 33 bp, synthetic construct
  misc_feature 1..33: note = SHR63422.1_as
  source 1..33: mol_type = other DNA
gtggtggtggtggtgttgtttgatccatccctg

SEQ ID NO: 15 - DNA, 33 bp, synthetic construct
  misc_feature 1..33: note = WP_066151830.1_s
  source 1..33: mol_type = other DNA
ggagatatacatatggaggtcgcggacacgact

SEQ ID NO: 16 - DNA, 33 bp, synthetic construct
  misc_feature 1..33: note = WP_066151830.1_as
  source 1..33: mol_type = other DNA
gtggtggtggtggtgcttaatccaaccagggct

SEQ ID NO: 17 - DNA, 33 bp, synthetic construct
  misc_feature 1..33: note = WP_066052166.1_s
  source 1..33: mol_type = other DNA
ggagatatacatatggatgaaaccgtaacgaca

SEQ ID NO: 18 - DNA, 33 bp, synthetic construct
  misc_feature 1..33: note = WP_066052166.1_as
  source 1..33: mol_type = other DNA
gtggtggtggtggtgttgtttgatccaaccttg

SEQ ID NO: 19 - DNA, 33 bp, synthetic construct
  misc_feature 1..33: note = WP_064202059.1 (WP_088909523.1)_s
  source 1..33: mol_type = other DNA
ggagatatacatatggagggcggtgagcaaacg

SEQ ID NO: 20 - DNA, 33 bp, synthetic construct
  misc_feature 1..33: note = WP_064202059.1 (WP_088909523.1)_as
  source 1..33: mol_type = other DNA
gtggtggtggtggtgttgcttgatccaacctgg

SEQ ID NO: 21 - DNA, 33 bp, synthetic construct; identical to SEQ ID NO: 20
  misc_feature 1..33: note = WP_108533520.1_s
  source 1..33: mol_type = other DNA

SEQ ID NO: 22 - DNA, 33 bp, synthetic construct
  misc_feature 1..33: note = WP_108533520.1_as
  source 1..33: mol_type = other DNA
gtggtggtggtggtgcttgatccaaccctgcgg

SEQ ID NO: 23 - DNA, 33 bp, synthetic construct
  misc_feature 1..33: note = WP_047973383.1_s
  source 1..33: mol_type = other DNA
ggagatatacatatggaggtcacagacacgact

SEQ ID NO: 24 - DNA, 33 bp, synthetic construct
  misc_feature 1..33: note = WP_047973383.1_as
  source 1..33: mol_type = other DNA
gtggtggtggtggtgtttgatccatccctgtgg

SEQ ID NO: 25 - DNA, 33 bp, synthetic construct
  misc_feature 1..33: note = ATN45517.1_s
  source 1..33: mol_type = other DNA
ggagatatacatatggaggacactgattcacct

SEQ ID NO: 26 - DNA, 33 bp, synthetic construct
  misc_feature 1..33: note = ATN45517.1_as
  source 1..33: mol_type = other DNA
gtggtggtggtggtgttttatccaaccttgtgg

SEQ ID NO: 27 - DNA, 33 bp, synthetic construct
  misc_feature 1..33: note = OV191_BI_s
  source 1..33: mol_type = other DNA
ggagatatacatatggaaaaaaaaaatccgcaa

SEQ ID NO: 28 - DNA, 33 bp, synthetic construct
  misc_feature 1..33: note = OV191_BI_as
  source 1..33: mol_type = other DNA
gtggtggtggtggtgattgatcgagcctggagc

SEQ ID NO: 29 - DNA, 33 bp, synthetic construct
  misc_feature 1..33: note = OV191_IS_s
  source 1..33: mol_type = other DNA
ggagatatacatatgaaagcgccgactacgtct

SEQ ID NO: 30 - DNA, 33 bp, synthetic construct
  misc_feature 1..33: note = OV191_IS_as
  source 1..33: mol_type = other DNA
gtggtggtggtggtggccgaaatcgcggatttc

SEQ ID NO: 31 - DNA, 33 bp, synthetic construct
  misc_feature 1..33: note = LL01_IS_s
  source 1..33: mol_type = other DNA
ggagatatacatatgagctctaactggaatatt

SEQ ID NO: 32 - DNA, 33 bp, synthetic construct
  misc_feature 1..33: note = LL01_IS_as
  source 1..33: mol_type = other DNA
gtggtggtggtggtgccttaaagatctaccgta

SEQ ID NO: 33 - DNA, 1326 bp, Bacillus sp. SD33
  source 1..1326: mol_type = genomic DNA
atgaaaactcgtaacaaatcgaaattgaaaaagctggttttgacagccgttgttgctgccaattgcctgtcagtatcaactgcattcgcagcggaaattagtacagattacacttccgtctggtcacgtcagcaagcagaaaaagtaacgcctactgacaaaacaacagcaccgaaaattgatcttgattttgatcttgtagcacctgatcaatgggtatgggatacatggccattacaaaatagagatggttcaatggcgattgtcaatggctaccgagtggcttttgcattggtagcaccgcgttctttaggatggggtgagcgccatacagaagcaagaattggaatgttctactccaaaaacggcaaagattggacgtacgcaggaatcccttatgactataataaagccttggggcatatgcaatgggccggaacagcaatgcttgatgacaatggaaaagttcatttattctatacggcaaccggtgaaaaaacaaattgggataacaatggatgggataaaagagccgtacagcggattgcgaaaacaacctttgatattcatacggataaaaacggggttcatctgaccaatgaagggaaacatcaagtcattcttgaagcagatggaaaatattacgagacacttgcacaagccaatagtccgatcattacggcattccgtgatccattcttcttccaggatccgaatacaggcaaagagtatattatcttcgaaggacaagctggaagtgatagagactttatcaaaccggaaaatatcggggatgaagaataccgtaaaacccattccgttcctgcaggagccgaattgtataacggtaatatcgggatcgcagaagtacttgacaaagacgtaaccaaattaaagcttctcccgccattgcttgagtcggttggaaccaatcaccagatggaacgtccgcacatggtcgtaaatggagatgattattatctatttaccatcagccatacctttacgtatgctcctggcctgactggtcctgatggtgtctatggatttgttggtaaaggactgttcggcagccataaaccaatgaatgaaagtggtcttgtgattgcgaatccaaaggaaagcccttatcaagcctattcttggatggttcttccagaccagcaggtaatcagctttattaacgagccgaaagatgagaacggtaatgtgaaatttggcggtacattcgccccaactctaaaagtgaagctgaatggcgaaacatctgaagttgtaaaagagggtaaagcgggcgaaattaaaccatttggggcaaatcgctaa

SEQ ID NO: 34 - protein, 441 aa, Bacillus sp. SD33
MKTRNKSKLKKLVLTAVVAANCLSVSTAFAAEISTDYTSVWSRQQAEKVTPTDKTTAPKIDLDFDLVAPDQWVWDTWPLQNRDGSMAIVNGYRVAFALVAPRSLGWGERHTEARIGMFYSKNGKDWTYAGIPYDYNKALGHMQWAGTAMLDDNGKVHLFYTATGEKTNWDNNGWDKRAVQRIAKTTFDIHTDKNGVHLTNEGKHQVILEADGKYYETLAQANSPIITAFRDPFFFQDPNTGKEYIIFEGQAGSDRDFIKPENIGDEEYRKTHSVPAGAELYNGNIGIAEVLDKDVTKLKLLPPLLESVGTNHQMERPHMVVNGDDYYLFTISHTFTYAPGLTGPDGVYGFVGKGLFGSHKPMNESGLVIANPKESPYQAYSWMVLPDQQVISFINEPKDENGNVKFGGTFAPTLKVKLNGETSEVVKEGKAGEIKPFGANR

SEQ ID NO: 35 - DNA, 1341 bp, Bacillus sp. SD33
  source 1..1341: mol_type = genomic DNA
atgaccgttatgaataagaaagcagtgtctgccatcgtcttggcggcgagtgttatagcctcaactttttccggggtttctgtaaaagcagaagacgtagggcaaacgacaaattggacacgggaacaggtctcaaaaattgaacttaatcaagataataccttgccttatacggatataagcaagcttaagaaattatcaccagattatcatatttgggacacgtggcccctgttggatcgcgatggaaatatcgcttcagtaaaaggctggaaagtgatgtttgccctatccgctccaaataatgtgctgcctggaaaagtacatgacattgcaaccatccgctatttttactcgaaaaatggtaaggattggactctcggcgggacacttttcccagaaggagcttcattaggttctcgcgaatgggctggatctgccatggtcgataatgggaaaattcatgccttctatacagcaactggccatagaggggaagagcgattgacatttgagcagcgcattgctgaggcatccggtgatattattgctgatagcaatggagttcattttgaaaattggggcaaacacaagatcattttagagccggacggtaaatattatcagacgaaggaacaagctcagcaaggcgaaggcggcggctacgctttccgtgatccgatgtggtttaaggacccaaaaaccgataaggaatatattttatttgaaggaaattcaggcggtactgtaggggagcgcacatttaaacaagaatatgccggaagttccgagtatacaagcaataacccggtacctgcgggagctgttcatgccaatgcgaacattggtatcgcagaggtagtggatggtaatccttctaaacttaaaatgctgcctcctcttttggaagcaaattatgtcaacgaagaattggaacgcccgcatattgtagtaaaggataaaaaatattatctctttactgacagccatatcaataaatatgctgaagggctgcaaggacctgaagggatgtatggatttgtttctgataacttgattggtggttatcagccgctgaataagagtggtttggttttagccaatcctccaggaaacccataccaagcgtattcatggcttgtccttcctaatttgaatgtcgtcgggtttgctcattttggcgatttaggcaacatgtcaattggtgatgttggaaaccaatcaccagaattccaatttagccattttggaggcacattggcgccaacgatacagctatcaatcaaaggcgacacaacaaaaatagcaaaagagttaagccctggctggattaaacaataa

SEQ ID NO: 36 - protein, 446 aa, Bacillus sp. SD33
MTVMNKKAVSAIVLAASVIASTFSGVSVKAEDVGQTTNWTREQVSKIELNQDNTLPYTDISKLKKLSPDYHIWDTWPLLDRDGNIASVKGWKVMFALSAPNNVLPGKVHDIATIRYFYSKNGKDWTLGGTLFPEGASLGSREWAGSAMVDNGKIHAFYTATGHRGEERLTFEQRIAEASGDIIADSNGVHFENWGKHKIILEPDGKYYQTKEQAQQGEGGGYAFRDPMWFKDPKTDKEYILFEGNSGGTVGERTFKQEYAGSSEYTSNNPVPAGAVHANANIGIAEVVDGNPSKLKMLPPLLEANYVNEELERPHIVVKDKKYYLFTDSHINKYAEGLQGPEGMYGFVSDNLIGGYQPLNKSGLVLANPPGNPYQAYSWLVLPNLNVVGFAHFGDLGNMSIGDVGNQSPEFQFSHFGGTLAPTIQLSIKGDTTKIAKELSPGWIKQ

SEQ ID NO: 37 - DNA, 4199 bp, Bacillus sp. SD33
  source 1..4199: mol_type = genomic DNA
attgaagaggtgcagtcacttcgaagagaagaactgtcatccgcccaaaatgttacaatggatgaagcaaataaacagcttcgaaaaatcaaaagcgatcaattcgaaatcgagttggaattcgatgtttccaatacgaaagcagccggtttaaaaatattaaaagacccaaatgaacaggaagaaaccagtattttttatgataatgaaaggaaaaccattcatattgaccgccagcgttcaagtaaaaatcctgaaattgaaaagggaattcaaggtggtgcgctaaaccttgaagacgatatcttaagggtacgcctatttgttgataaatcgattgtggaagcatacgtcaataatgaaataagtatttcgtcccgtgtatttccaataatggatcaatcgaaaggactcgaagtatttggagtggatggagaaccatttatacgttcgatgagggtatggagtatggctacagccattgaaggagagaaagattagccttacgggtttaactctatctaatgagttttgtattggttatatgaaaatataactagtaaatcctaatgaaattaagggtatattatcctattgtaggaaattgtcgaacagaatataatgttccctgtaaacaaaattatgcgggattgtgactggtaaagcaggcaagacctaaagtgtatgaagggcgaagtgtacctttttggtagacgtacccttgtacattttaggtctttttttgttctctgagaaaggattttaactagtttgaatagacgaaaaattcttaacggacacaatgttcccgcgaaaaatggaggatttaggggaaatggaaatgaaaactcgtaacaaatcgaaattgaaaaagctggttttgacagccgttgttgctgccaattgcctgtcagtatcaactgcattcgcagcggaaattagtacagattacacttccgtctggtcacgtcagcaagcagaaaaagtaacgcctactgacaaaacaacagcaccgaaaattgatcttgattttgatcttgtagcacctgatcaatgggtatgggatacatggccattacaaaatagagatggttcaatggcgattgtcaatggctaccgagtggcttttgcattggtagcaccgcgttctttaggatggggtgagcgccatacagaagcaagaattggaatgttctactccaaaaacggcaaagattggacgtacgcaggaatcccttatgactataataaagccttggggcatatgcaatgggccggaacagcaatgcttgatgacaatggaaaagttcatttattctatacggcaaccggtgaaaaaacaaattgggataacaatggatgggataaaagagccgtacagcggattgcgaaaacaacctttgatattcatacggataaaaacggggttcatctgaccaatgaagggaaacatcaagtcattcttgaagcagatggaaaatattacgagacacttgcacaagccaatagtccgatcattacggcattccgtgatccattcttcttccaggatccgaatacaggcaaagagtatattatcttcgaaggacaagctggaagtgatagagactttatcaaaccggaaaatatcggggatgaagaataccgtaaaacccattccgttcctgcaggagccgaattgtataacggtaatatcgggatcgcagaagtacttgacaaagacgtaaccaaattaaagcttctcccgccattgcttgagtcggttggaaccaatcaccagatggaacgtccgcacatggtcgtaaatggagatgattattatctatttaccatcagccatacctttacgtatgctcctggcctgactggtcctgatggtgtctatggatttgttggtaaaggactgttcggcagccataaaccaatgaatgaaagtggtcttgtgattgcgaatccaaaggaaagcccttatcaagcctattcttggatggttcttccagaccagcaggtaatcagctttattaacgagccgaaagatgagaacggtaatgtgaaatttggcggtacattcgccccaactctaaaagtgaagctgaatggcgaaacatctgaagttgtaaaagagggtaaagcgggcgaaattaaaccatttggggcaaatcgctaatgataactcgaaaaggagaaagaaggatgaccgttatgaataagaaagcagtgtctgccatcgtcttggcggcgagtgttatagcctcaactttttccggggtttctgtaaaagcagaagacgtagggcaaacgacaaattggacacgggaacaggtctcaaaaattgaacttaatcaagataataccttgccttatacggatataagcaagcttaagaaattatcaccagattatcatatttgggacacgtggcccctgttggatcgcgatggaaatatcgcttcagtaaaaggctggaaagtgatgtttgccctatccgctccaaataatgtgctgcctggaaaagtacatgacattgcaaccatccgctatttttactcgaaaaatggtaaggattggactctcggcgggacacttttcccagaaggagcttcattaggttctcgcgaatgggctggatctgccatggtcgataatgggaaaattcatgccttctatacagcaactggccatagaggggaagagcgattgacatttgagcagcgcattgctgaggcatccggtgatattattgctgatagcaatggagttcattttgaaaattggggcaaacacaagatcattttagagccggacggtaaatattatcagacgaaggaacaagctcagcaaggcgaaggcggcggctacgctttccgtgatccgatgtggtttaaggacccaaaaaccgataaggaatatattttatttgaaggaaattcaggcggtactgtaggggagcgcacatttaaacaagaatatgccggaagttccgagtatacaagcaataacccggtacctgcgggagctgttcatgccaatgcgaacattggtatcgcagaggtagtggatggtaatccttctaaacttaaaatgctgcctcctcttttggaagcaaattatgtcaacgaagaattggaacgcccgcatattgtagtaaaggataaaaaatattatctctttactgacagccatatcaataaatatgctgaagggctgcaaggacctgaagggatgtatggatttgtttctgataacttgattggtggttatcagccgctgaataagagtggtttggttttagccaatcctccaggaaacccataccaagcgtattcatggcttgtccttcctaatttgaatgtcgtcgggtttgctcattttggcgatttaggcaacatgtcaattggtgatgttggaaaccaatcaccagaattccaatttagccattttggaggcacattggcgccaacgatacagctatcaatcaaaggcgacacaacaaaaatagcaaaagagttaagccctggctggattaaacaataaggaaatgatttgaccggttcccgcactccaatcgctcactaagagaccgtataagcgctcgtggaaccggttcctgagctctaatcgggcgcttgaaatttatggttaatcaacaaagtttttaacaaagcaaaagtaagaaggcatttgggggaacacttttcatgaaatggaacaaagttaaaaaaagcaaatctatcatagcagctattatcggactttttattatcttcatacccattgttggtccaaccgtttctgcccaagaaaatgcagatacattcaactggaccagagaaaatgttagcactctaacaatcaatgagcaaaatacagctccgacatttaataaagatgagctcgttaaactttcatcagactattatatttgggatgcatggccattgcaggatttgaacggtcatccagctgtagtaaatggtttcaaaattattttcgccctatcggtaccgaaggatgtccttcctggaaaacgccatgatctagctcaaattcaatatttctattcaaaagacggaaagagctgggtgtcaggtggtcccgtttttaaagatggagatgcattgggatccagacagtgggctggctcatccatcattaatcgagatgggagattacaaatcttttacacagcaacagggcaa

SEQ ID NO: 38 - DNA, 1248 bp, synthetic construct
  misc_feature 1..1248: note = Bacillus onubensis (WP_099354679.1)
  source 1..1248: mol_type = other DNA
gcagaaacagaggtaacgacaaattggacaagagaacaggcgtcaaatattgaacttaatcaagataatactttaccttatacagatataagtgaattagagaaattagcaccagattatcatatttgggatacttggccactaactgatcgtgatggaaatatcgcatctgttaaaggatggaaagtgttgtttgcattatcagcaccaaatgatgtacttccaggtaaagtacatgatatcgcaacaatccgctatttttattcgaaaaatggtaaagattggacacttggcggaacacttttcccagaaggagcttcattaggttctcgtgaatgggctggttctgcaatgatggatgatgggaaaattcatgcattttatacagcgactggacatagaggacaagagcatttaacttttgaacagcgattagcaatggctacaggtgatatcattgccgatagcaatggagttcactttgaaaactggggtgatcacaagatcattttagaaccagatggtaaatattatcaaacaaaagagcaagcacagcaaggtgaaggcggaggctatgctttccgtgatccaatgtggtttaaagacccaaaaactgataaggaatatattctgtttgaaggtaattcaggcggtgctgtaggtgaacgcacatttaaacaagaatatgcaggaagtactgagtacacaagtgaaaatccagttcctgcaggtgctgtacatgcgaatgccaacatcggtatcgcagaggtagttgatggtgatccttcaaatcttaaaatgcttccaccacttttggaagcaaattatgtaaatgaagaattagaacgtcctcacatcgttgtaaaggataaaaaatattatcttttcacagatagccatatcaataaatatgctgaagggcttcaaggtcctgaaggtctttatggttttgtttctgatacattaatcggtggttatgagccgttgaatgaaagtggtttagttttagcaaatcctcctgaaaatccatatcaagcatattcatggcttgttcttccgaacttaaatgtagtagggtttgctcattttggagatttaggtgatatgtcaattggtgatgtaggaaaccaatcaccagaattccaatttgaacattttggtggaacgttagctctaacagttaagctatcaatcaaaggcaatactacaaaaatagtaaaagaatatagccctggttggattaagcaa

SEQ ID NO: 39 - DNA, 1248 bp, synthetic construct
  misc_feature 1..1248: note = Mycobacteroides abscessus subsp. abscessus (SHR63422.1)
  source 1..1248: mol_type = other DNA
gatgaaaccgtaacgaccaccaattggacaagggaacaggcttcaaaaattgaactgaatcaagatagtaccttgccatatacggatatctctgaattggagaaattcgcacctggttatcatgtatgggattcatggcctttaaccgaccgcaacgggaatattgcttccgttaaaggctggaaggtattgtttgctctttcagctccagacaatgttctacccggtaaagtgcatgatattgcgaccattcgttacttttactcgaaaaatggaaaggattggacgctagggggaacacttttcccagaaggagcatcactaggttcacgtgaatgggcaggatctgccatgatggatgatggaaaaattcatgccttctatacagcaaccggtcatagaggagaagctccgctgacgtttgaacagcgtctggcgatggctacaggtgatatcgtagctgacagtgagggtgtccgttttgaaaactggggagatcacaagatcattctagagccagatggagagcactatcaaacgaaggagcaggcacagcaaggtgaaggaggcggctatgctttccgtgatccgatgtggttcaaggatccaaagacagaaaaagaatacattctgtttgaaggtaattcaggtggtgcagtaggggaacgtacatttaagcaggagtacgcgggaagcacggagtatacggataagaaaccagtgccagctggagctgtccatgccaatgccaatattggaatcgcagaagtggtggatggaaatccttccaacctgaagatgcttccaccgcttttggaagcaaattatgtaaatgaagagctagagcgaccacatatcattgtgaaggataaaaaatattatctgttcaccgacagtcatatcaataaatatgcggaaggactacaaggaccagaagggctgtatggatttgtgtctgatacgttgacgggtggatatgagccacttaatggtagtggactagtcatggccaatcctccggaaaatccttaccaggcgtattcatggcttgtccttccgaatttgaatgtcgtaggattcgcccactttggtgatttaggtaacctgtctattggcgatgttggaaaccaggaacctgagttccagttcagccattttggcggtacactagctccgacagtaaaaatatccatcaatggatcgacaaccaagattgaaaaagaattcagccagggatggatcaaacaa

SEQ ID NO: 40 - DNA, 1245 bp, synthetic construct
  misc_feature 1..1245: note = Bacillus krulwichiae (WP_066151830.1)
  source 1..1245: mol_type = other DNA
gaggtcgcggacacgactgttaactggactcgtgaacaagtatcgaaaattgaactcaataaagataataccttgccttatacagatgtaagtaaactagagaaatttacggaagattaccatgtttgggattcatggccactaaccgaccgcgatggaaatatcgcctcgattaaaggctggaaagtgttgtttgcactgtctgctcctaacaatgtactgccaggtaaagtgcatgacattgcaaccatccgctatttttattcgaaaaacgggaaagattggacgcttggtggaacgcttttccctgagggagcttcattaggatctcgtgaatgggctggatctgccatgatggatgacggtaaaatccatgcattctatacagcaactggacatagaggtcaagagcatttaacttttgaacagcgattggcgatggctacaggtgatatcgtagcagacagcaaaggagtccgttttgaaaactggggtgatcacaagatcattttagagccggacggtaagtattatcaaacaagagagcaagctcagcaaggtgaaggcgggggctatgctttccgtgaccctatgtggtttaaagaccccaaaacggacaaggaatatattttgtttgaagggaattcaggcggtgctgtaggtgatcgtacctttaaacaagaatatgcaggaagtattgagtacactagtaaaaacccagttcctgcaggcgctgtacatgcgaatgggaacatcggtattgcagaggtagtggatggcgatccttcaaatcttaaaatgctcccgccgcttttggaagctaattatgtaaatgaagaattagaacgtccgcatatcgttgtaaaggataataaatattatttattcactgatactcatatcaataaatatgctgaagggcttcaaggtcctgaaggtttgtatggttttgtttctgatacattgttcggtggttatgagccgttaaatgaaagtggtttagttttagctaatcctcctgaaaatccataccaagcttattcatggttggttcttccgaatttaagtgtcgtagggtttgctcattttggtgatattggtgatatgtcaattggtgatattggacatcaaccagatgaattccaatttgaacattttggaggaacattgcctccaactgttaagctatcaatcaaaggcgatacgacaaaaataggaaaagaatacagccctggttggattaag

SEQ ID NO: 41 - DNA, 1248 bp, synthetic construct
  misc_feature 1..1248: note = Bacillus korlensis (WP_066052166.1)
  source 1..1248: mol_type = other DNA
gatgaaaccgtaacgacaaccaattggacaagggaacaagcttcaaaaatagaattgaatcaagataataccttgccatatacggatatctcgaagttggagaaatttgcacctggttaccatgtttgggattcatggcctttaaccgaccgtgatgggaatattgcttccattaaaggctggaaggtattgtttgctctatcagctccagacaacgtgctaccaggtaaagtccatgatattgcaaccattcgttatttttactcaaagaacggaaaggattggacgcttggcgggactctcttcccagaaggagagtcactgggttcacgcgaatgggcaggatctgccatgatggatgatggcaaaattcatgccttctatacagcaacaggccatagaggagaagctccgcttacgtttgaacagcgattggcaatggcaacagccgatatcgtagctgacagcgagggtgtccgttttgaaagctggggagatcataagatcatcatggagccagatggcgtacactaccaaacgaaggaacaggcacagcaaggagaaggaggcggctatgctttccgtgatccgatgtggttcaaggatccaaaaacagaaaaggaatacattctgtttgaagggaattctggcggtgcagtaggggagcgtacattcaagcaggagtatgctggaagcaccgaatacacggataaaaatccagtaccagcaggtgcagttcacgcaaatgccaatattggaattgcagaggttgtgaatggagatccttcaaacctgaagatgcttccgccgcttttggaagctaattatgtaaatgaagagctggaacgtccacatatccttgtgaaggataaaaaatattacctattcacagacagccatatcaataaatatgctgaaggactacaaggaccagaaggactgtatgggtttgtgtctgatacattgactggcggatatgagccgcttaatggaagtgggctggtcatggccaatcctccagaaaatccttaccaggcctattcatggcttgtccttccgaatttgaatgtggtaggattcgcccactttggtgatttaggtaacatgtcaattggcgatgttggaaaccaggatccggaattccaattcagccattttggcggtacaatatctccaactgtgaaactatcaatcaatggatcgacaacaaagatcgagaaagaattcaaccaaggttggatcaaacaa

SEQ ID NO: 42 - DNA, 1248 bp, synthetic construct
  misc_feature 1..1248: note = Brevibacillus brevis (WP_064202059.1)
  source 1..1248: mol_type = other DNA
gagggcggtgagcaaacggtcaactggacccgcgagcaggcatcgaaaatcgagctgaatcaagacaataccttgccgtacactgacatcagcaaactggaaaaattggcgccgggctatcacatgtgggatacgtgggcactgacagaccgtgacgggaatgtagcctcgatcaaaggctggaaagtgatattcgcgcttaccgcaccgagtgatgtgctgccgggcaaagtgcacgacattgccacgatccgttacttttattcgaaaaacggaaaagattggacgctgggtggcgagctgttcccgagcggatccgcgctcggttcccgccagtgggctggatcggctatgatggataacggcaaaatccatgcgttctacaccgcaaccggacacaaaggtgaagagcgtttgacctatgaacaacgtttggccatggctaccggcgatatcgtcgcggacaacagcggagtccgattcgaaaattggggcgatcaccgcatcattttggagccggacggaaaacactatcagaccaaagaacaagcgcagcagggtgaaggcgggggttacgctttccgcgatccgatgtggtttaaagatccgcaaacgaaaaaagaatacctgctgtttgaagggaattccggaggcaccgcagccgaccgcaagttgaaaccggaatatgtcggaagccctgagtttgcagggcagcaaaacgtgcctccaggtgccgtacacgctaatggtaacattggcattgctgaggtggtaggtggcgatttttccaaaattaaaatgcttcctccgctcgtagaagccaactacgtaaatgaagaactggagcgcccgcatattgtggtgaaggataaaaagtattatctgtttaccgacagccacatcaataaatatgcggatggactcaccggaccggacggactgtacggattcgtttcagacaagctgatcggcggatataaaccgctgaacggaagcggtttggtcttggccaatccggcggataatccataccaagcatattcctggttggtgcttccgaacttgaacgtggtcggtttcgcccattttggcgatctgggcaacatgtccatcggcgatgtcggcaatcagactccggaattccaattcagccactttggtggcacattggctccaacagtgaagctgtcgatcaaagacgatcgcacaaaattggaacaagagtacgagccaggttggatcaagcaa

SEQ ID NO: 43 - DNA, 1248 bp, synthetic construct
  misc_feature 1..1248: note = Brevibacillus formosus (WP_088909523.1)
  source 1..1248: mol_type = other DNA
gagggcggtgagcaaacggtcaactggacgcgcgagcaggcatcgaaaatcgagctgaatcaagacaataccttgccgtacaccgacatcagcaaattggaaaaattggcgccgggctatcacatgtgggatacgtgggcactgacagaccgtgacgggaatgtagcctcgatcaaaggctggaaagtgatattcgcgcttaccgcaccgagtgatgtgttgccgggcaaagtgcacgacattgccacgatccgttacttttattcgaaaaacggaaaagattggacgctgggtggcgagctgttcccgagcggatccgcgctcggttcccgccagtgggctggatcggctatgatggataacggcaaaatccatgcgttctacaccgcaaccggacacaaaggcgaagagcgtttgacctatgaacaacgtttggccatggctaccggcgatatcgtcgcggacaacagcggagtccgattcgaaaattggggcgatcaccgcatcattttggagccggacggaaaacactatcagaccaaagaacaagcacagcagggtgaaggcggtggttacgctttccgcgatccgatgtggtttaaagatccgcaaacgaaaaaagaatacctgctgtttgaagggaattccggaggctctgctgccgaccgcaagttgaaaccggaatatgtcggcagtcctgaatttgccgggcagcaaaacgtgcctccaggtgctgtacacgctaatggcaacatcggcatcgctgaggtggagggcggcgatttttccaaaatcaaaatgcttcctccgcttgtagaagccaactacgtaaatgaagaactggagcgcccgcatattgtggtgaaggataaaaagtattatctgtttaccgacagccacatcaataaatatgcggatggactcaccggaccggacggactgtacggattcgtttcagacaagctgatcggcggatataagccgctgaacggaagcggtttggtcttggccaatccggctgataatccataccaagcatattcctggttggtgcttccgaacttgaacgtggtcggtttcgcccattttggcgatctgggcaacatgtccatcggcgatgtcggcaatcagactccggaattccaattcagccactttggcggaacattggctccgacggtgaagctgtcgatcaaagacgatcgcacaaaattggaacaagagtacgagccaggttggatcaagcaa

SEQ ID NO: 44 - DNA, 1245 bp, synthetic construct
  misc_feature 1..1245: note = Paenibacillus elgii (WP_108533520.1)
  source 1..1245: mol_type = other DNA
caggggggagaacagacagtcaactggacccgggaagacgtctcgaaaatcgaactgaatcaagataatacgttgccttacatcgatgtaagcaagctggaaaagatggctcccggctaccacatctgggatacgtggccgctgctggaccgcgacgggaacatcgcatcctacaaaggctggaaagtgatcttctcgctttccgccccgaatactgttcttcccggcaaagtgcacgatattgcgacgatccgctacttctactcgaagaacggcaaagactggaccctgggcggcgaattgttcccagcgggaacagcgctcggccagcgccaatgggccggttcggcgatgctcgacggcgatcaaattcacgccttctacaccgcgaccggacgggagggccaggctcagcttacctacgagcagcgcattgccagcgccgcgggccgtattgtggccgacagcaccggcgtacgcttcgagaactgggggcagcaccgcgttattctggaaccggacgggaaatactaccagaccaaagagcaagcgcagcaaggggaaggcggcggctatgcgttccgcgacccgatgtggttcaaagacccgaaaacgggcaaagaatatttgctcttcgaaggcaactccggcggcgctgttggggagcgaagcttcaagcccgaatacgccggaagcggggagtatcttcaacagcatccggtgccggccggcgccgtgcacgctaacggcaacatcggcatagccgaagtggtgaacggcgatttgacgaacgttaagctgcttccgccgctgattgaagcgaactatgtgaacgaagagctggaacgtccgcatgtggtcgtcaaagacaagaagtattacctgttcaccgacagccatatcaacaaatacgctgaggggacgcatggaccggaaggaatgtacggattcgtctccgacaagttgatcggcggttacaagccgcttaatggaagcggcctggtcctggctaatcccccggaaaatccgtaccaagcctattcctggttggtcacgccggaactgaatgtagtgggattcgctcatttcggcgatctggacaacctaacgattggcgatgtaggcaaccaatctccggaattccagttcagccacttcggaggcacgttggcgccgacggtaaagatttccattaaaggggatcgaacgcagatcgaaaaggttctgccgcagggttggatcaag

SEQ ID NO: 45 - DNA, 1233 bp, synthetic construct
  misc_feature 1..1233: note = Bacillus sp. LL01 (WP_047973383.1)
  source 1..1233: mol_type = other DNA
gaggtcacagacacgactgttaactggactcgtgaacaagcttcgcaaatcaagttagataaaagcaataccctgccatatacggacatcaaggagttagaaaagatgacgtctgactatcacatttgggactcgtggccactgactgaccgcgacggtaatatcgcgagagttaaaggctataaagtgctctttgcactaactgcaccaagtgatgtgctgccgggtaaagtccacgacatcgctaaaattcaatacttttattcccgtaacgggaaggactggacgctaggcggtgaactgttcccagatggagactcgcttggttcccgagaatgggcaggttcggctatgtttgataaaggtaaaatctacgctttctacacagcaacgggtagaaatggtgaagaaaggttaacgtatgagcagcgtatggcgatgtctataggtgacgttatcaccgataaagacggcgttaggtttgaaaattgggacgagcacagcattttatttgagccagacggtgagcactaccaatcttatgagcaagctatagagggcggatatagcggctatgcgttccgggatccacagtggtttaaagatcctaaaacgagcaaggaatatattgtttttgaaggtaactcaggcggagcggtttctgaacgtacgtgcaaacctgaatattatggcagccctgagcacacggcaccaaacggttctgaacacttcaacggcaacatcggcatttccgaagtggttaacggcgacttctctaacattaaaatgcttcctcctttaatagaggctaaatgtgtgaacgatgagttggagcgtccacatattattgtgaaggacgataagtattatctatttaccgacactcacattaataagtatgctccggggcttgaaggtccagaagggctatacggattcgtttcggacacgctaatcggaggatataagcccctgaacgggagcggacttgttatcgccaatcctccagaaaatccatatcaagcgtattcatggcttgtactgcctagtttagagattatctcttttgcgcattttggtgatctaggtgacatggatattaatgaggtcggccaccagtctccagaattccagttcgaacactggggtgggacgatggctccgaccgtagagatctctattgatggtgatcgtacggaaattaagagagaaagaccacagggatggatcaaa

SEQ ID NO: 46 - DNA, 1218 bp, synthetic construct
  misc_feature 1..1218: note = Salipaludibacillus agaradhaerens WDG185 (ATN45517.1)
  source 1..1218: mol_type = other DNA
gaggacactgattcacctgtcaactggacacgtgaacaagtggaccaaattgagttggatgagtccaataccataccatatacgaacattaaggaattggaaaaaatgacacctgactatcacatatgggattcgtggcctctgaccgaccgtaatggtaatgtcactgaagttaatggttggaaagtactctttacacttagtgctccgagtgatgtgttgccaggtaaagtgcatgacattgccaaaatccaatattttgtttcccgtgacgggaaagattgggagctaggcggcgagctgttccctgaagaggattccctcggttcaagggaatgggctggctcagctatgatggacgaagatgaaggtaaaatctacgcattctataccgcgactggtcgaagaggggaagaaaatcttacgtatgagcagcgtttggccatgtctgtcggtgatgtagtcgccgataaaaacggcgtccattttgaaaattgggatgaacatagtatcattcttgagccggacggtgaagactatcaatcatatgaacaagctatggagaatggatatagcggctatgcgtttcgtgatccacagtggttcaaagatacgaaaacggggaaggaatatattctgtttgaaggcaattcaggaggtcgcgtttctgaacgcacgtgtgaaaatgaagacgttccggaaggttctgagcacttcaatggtaatatagggattgctgaagtggccgacggtgatttttctgacttgaaagtgcatgctcctttattggaagccaattgtgtgaatgatgagttggagcgtccacatattattgtcaaagatgataagtactatctgtttactgatacgcacattaataaatatgcaccaggaattgaaggaccagaaggcctgtatggctttgtttccgatacactatttggtggttatgaacctttaaatggaagtgggctcgttttagccaatccaccagaaaacccgtatcaagcctactcttggttagtgttacccgatcttaaagtcatcgcttttgcgcaatttggtgatttggatggcatggacatcaatgagatcggccaccaggaccctgaattccaattcgaacattggggcggtacaatggctccgacgctggaaatcggtattgacggtgatcgtacggaatttaaaaaggaactaccacaaggttggataaaa

SEQ ID NO: 47 - DNA, 1260 bp, synthetic construct
  misc_feature 1..1260: note = Paenibacillus sp. OV191 (PYE68991.1 (OV191_BI))
  source 1..1260: mol_type = other DNA
gaaaaaaaaaatccgcaaacagaaataacaacgactaactggacacgcgagcaagcgtccagtatcgtacaaaacgaaaacaacaccctgccttattttgatatcaaaaagcttgaaaaaatgacgccggactatcacatctgggatacatggccgctgatggaccgcgacggaaatgttgctaattacaaaggctataaagtgctcttcgcgctttccgcaccgagcaacgtgctgccgggcaaagttcacgatatcgcaacgattcgttacttcatctcgaaagacggcaaggaatggaaatttgtaggcgacctgttcccggcaggcactaggctcggttcccgtaactgggcaggttccgcgatgctggacggcgataaaatccatgccttctacaccgctaccggccgtgaaggcgagaaaaacctgacttatgagcaacgcttggctatggccgtcggtgaaatcaaagccgacaaaaacggcgtaacattcacgaactgggctccgcaccgcatcattatggagccggacggccaatactaccaaacgctggagcaagcgaagcaaggtgaaggcggcggttacgctttccgtgatccaatgtggtttaaagatcctaaaacgaaaaaagagtacattgtattcgaaggccaatccgcaggcgctgttggcgaccgcgaattgaagccggaatacatcggcagcgaagagttccaaaaaactcatactgttcctgcaggagcagctagtgccaacgccagcatcggtattatcgaagttgttaaaggtgatttcaataatctgaagcttcttcctccgcttcttgaagcgaactatgtaaacgaagaactggagcgtccgcacatcgtagtgaagaacggtaaatactatctgttcacagacagccacatcaacaaatacgcggaaggtctgcaaggtcctgaaggcctgtacggtttcgtatccgacaaactgggcgaaggcttcaaaccgctgaatggcagcggtctggttctcgccaaccctaagaacaacccgtaccaagcttactcctggctggttctgccgaacctgaacgtcgttggcttcgcgcacttcggcgatttgggcacaatgtccattggagatgtcggcaatcagtctcctgaattccaattcgcacactggggcggaacgcttcctccgacggtccaaatcgcaatcaatggcgacacgaccaaaattacaggagaacttgctccaggctcgatcaat

SEQ ID NO: 48 - DNA, 1266 bp, synthetic construct
  misc_feature 1..1266: note = OV191_IS
  source 1..1266: mol_type = other DNA
aaagcgccgactacgtctgtgcctaacgattacacggccgtctggtcccgtcaagcagcagagaaagtcaagctttcacctacgaacacgtcacctaagattgacactaactttaaactggccgctcctgatgtatggatctgggatacttggccgctccaaaaccgcgatggctcccttgctatcgtcaacggatacagaatcgcattcgcattggtagctcctcgtacgttcggatggaacgaccgtcacaccgaagccagaatcggtatgttctactccaaggacggagtcgactggacttacgcaggcattccttatgactataataaagcttacggccacatgcagtgggccggttccgcaatgctggacaagaaaggcaaaattcacttgttctacacggctactaccgataagaacgctcacggcggcaaagagtgggatcagaacggctgggtacagcgcgctgaacaacgtctggccacaacgactttcgatattaaagcggataacagcggcgttaagctgatcaatgaaggcccgcaccaaatcatcgcccagccggacggcaagtattacgaaacaattgatcagttctacgatggaggccacaacatcacggctttccgcgatccgttcttcttccaggatccgaattcaggcaaagagtacatcatattcgaaggccaagtagccggcaaatcgagcgaacaaaaactgaagcctgagaacatcggtgacgaagcataccgcagcacgcataccgttccggatgaagcagcactgtatgacggtaacatcggtattgcggaagtactcgacaatgatgtgaccaaactgaaattgcttcctcctttgctggaatccatcggtgcgaaccatcaagtagaacgtccgcacatgtatatcaaaggcaacgattattacctgatgacaatcagccataccttcacatacgcaccaggcttgaccggtccggacggcgtatacggcttccacaacgaaggcggcgtccgcggcgattacaaaccgcttaacggttccggtcttgttgtagccaacccgaaagaaagcccgtaccaagcttactcctggatggttcttccggatgaaacggcaatcagcttcatcaatgaaccgcttgatgagaacggcaatgtgaaattcggcggtacattcgctccgacgctgcagctgtccttcgagggcgacaaaactaaaatcgtcggtgaattgcagcacggtgaaatccgcgatttcggc

SEQ ID NO: 49 - DNA, 1278 bp, synthetic construct
  misc_feature 1..1278: note = LL01_IS
  source 1..1278: mol_type = other DNA
agctctaactggaatattgaggatgattacactgcatcatggtccagacagcaagcagagaaagtggctctgacggaagagacgacagccccaatcatcgatttggactttgaagacgtagcaccggatgtgtgggtttgggatacgtggccgcttcaaaatagagacggttcccttgcgaacgtgaaaggttacagaatcgcattcgcattggttgcaccgcgtacttatacttggcatgaccgtcatactgaagcaagaatcggcatgttctactcaagaaacggcaaggattggacgtatgctggaattccatacgattatgacaaggcgttaggacacatgcaatgggctggttcagctatgttggatgaaaaaggaaaagtgcatttcttctatacagcaactactgatatgaatgccaatggcggtaaagaatttaataaagacggatgggtgcaaagagcggagcagcgactcgctaagacgacctttgatatcagtgcagataaaaatggtgttcatctgacgaatgaaggggctcaccaaattcttcttgaagcagacggtcatcattatgaaacgatcgaacagttccaagagcacggaaatatcatcactgggttccgcgatccgtttttcttcaaagatccgaatacaggcgaagaatacattatttgggaaggtcaggctggcgccaatagaaatgatatcaaaccggaaaatatcggggataaagaataccgcgaaacgcataacgttccggatcatgcgaaattttacaacggaaatattgggattgcaaaagtgcttgacaacgacgtaactaagctagaaatactaccgccacttcttgagtcggttggggttaaccatcagttagaacgtccgcatgttgtggtaaaagacgacacttactacttgcttacaatcagtcatgaatttacgtttgcaccaggtttaaccggtccggatggattgtacggatttgtcggcgagggaggcttgcgtacagattataagccagtcaacggcacaggtctcgtggttgccaatccagcagaaaaaccgtttcaagcttattcttggtgggcggctccagatggtcaggtcatcagcttcattaatgaacctgtagacgaaaatgggcaagttaaatttggtggaacatttgcaccgacgctgaaggtctcctttgacggtgataaaacaaagattgtgaaagaaatgcaagctggggaaatcaagccattcggtccttacggtagatctttaagg